European Patent Specification EP 3 715 463 B1, published January 25, 2023. Title: A Method of mass production of carbonic anhydrase in plant. Applicant: POSTECH ACADEMY-INDUSTRY FOUNDATION BioCompanion Inc. The sequence listing filed with the application follows.

SEQUENCE LISTING (13 sequences)

SEQ ID NO: 1 - protein, 287 aa, Artificial Sequence
  amino acid of GCCAHa3
MNFFATASVFLLFLSVALPVRANEEIEVDTAGCPVKSAQGDFSYDMTLPNNPTRWGDIKEDFATCKEGEKQSPINFPANVQYAPKSAGPKSQMSLANMTFGASSYNWAMSCSDESGSCGKTSFAGKTYELINVHFHSPSEHKLFGKEYPLECHMVHAAEDGSLAVVGMMFEYAEQTSYPARIYQNVVEEYGDNVVFSTILGGVKSDRGEWAVPVGQLVNHNKGYCSYSGSLTTPPCTESVTWFMSMNIWTVSERQVHDYVRTVGTSIEGNHRPVQPLNERPVTCYVS

SEQ ID NO: 2 - DNA, 864 bp, Artificial Sequence
  GCCAHa3
atgaacttcttcgctaccgcctccgtctttctactcttcttgtccgtcgccctccccgtgcgggcgaacgaggaaatcgaggtcgacaccgccggctgccccgtcaagagcgcccaaggagacttcagttatgacatgactcttccaaacaaccccacccgctggggcgacatcaaggaggacttcgccacatgcaaggaaggagaaaagcaatcgcccatcaacttccccgccaacgttcaatacgccccgaaatcggccggacccaagtctcaaatgtcgctcgcaaacatgacctttggcgcctcctcctacaactgggccatgtcctgcagcgacgaatccggatcgtgtggaaagacctccttcgctggaaagacctatgaacttatcaatgttcacttccactccccgagtgagcacaagttgttcggcaaagaatatccgcttgaatgtcacatggtgcatgctgccgaggatggatcgcttgctgtggtcggaatgatgtttgagtacgccgaacaaacctcctatcccgccagaatttaccagaacgtcgttgaggaatatggcgacaacgtcgtcttttccactattttgggaggcgtcaagagcgatcgtggagaatgggctgtgccggtgggtcaactggtcaaccataacaagggatattgctcctactccgggtcgctcaccacaccgccttgcactgaaagtgtcacctggttcatgtctatgaacatctggaccgtgtctgaacgacaggtgcatgactacgtccgaacggttggcaccagcattgagggaaatcatcgaccggttcaaccactcaacgaacgtccggtcacttgctacgtgtcctaa

SEQ ID NO: 3 - DNA, 27 bp, Artificial Sequence
  5 UTR
tctagaattattacatcaaaacaaaaa

SEQ ID NO: 4 - DNA, 273 bp, Artificial Sequence
  BIP
atggctcgctcgtttggagctaacagtaccgttgtgttggcgatcatcttcttcggtgagtgattttccgatcttcttctccgatttagatctcctctacattgttgcttaatctcagaaccttttttcgttgttcctggatctgaatgtgtttgtttgcaatttcacgatcttaaaaggttagatctcgattggtattgacgattggaatctttacgatttcaggatgtttatttgcgttgtcctctgcaatagaagaggctacgaagttaa

SEQ ID NO: 5 - protein, 60 aa, Artificial Sequence
  M DOMAIN (AMINO ACID)
ANITVDYLYNKETKLFTAKLNVNENVECGNNTCTNNEVHNLTECKNASVSISHNSCTAPD

SEQ ID NO: 6 - DNA, 230 bp, Artificial Sequence
  M DOMAIN
ggatcccgatggcaaacatcactgtggattacttatataacaaggaaactaaattatttacagcaaagctaaatgttaatgagaatgtggaatgtggaaacaatacttgcacaaacaatgaggtgcataaccttacagaatgtaaaaatgcgtctgtttccatatctcataattcatgtactgctcctgatggtggaggaggttctggtggtggatcaactagtcatatt

SEQ ID NO: 7 - DNA, 240 bp, Artificial Sequence
  SUMO
aatttgaaagtgaagggacaggacggaaacgaggttttcttccgtatcaaaagatcaacacaactcaagaaactcatgaatgcttactgcgatagacaaagcgtggacatgacagctatagctttcctatttgatgggagaaggttgagagcggaacagactccggatgagcttgaaatggaagatggagatgagattgacgcaatgttacatcagactggtgccggcggtcccgggggt

SEQ ID NO: 8 - DNA, 498 bp, Artificial Sequence
  CBM3
ggaggaggttcaggtggtaccgtatcaggtaaccttaaggtggagttttacaactcgaacccttctgatacaactaactcaataaacccacagttcaaagttacaaacacaggcagctctgcgatcgatttgtctaaattaaccctcagatactattatacggttgatggacagaaggaccagactttctggtgtgatcatgcagctatcattggttctaacggtagctacaacggaattacatcaaacgtgaagggcactttcgttaagatgtcctctagcactaacaacgcagacacatatttggagatcagttttacggggggaacccttgaaccaggtgctcacgtccagattcaaggaagattcgctaaaaacgactggtcgaactatacccaaagtaatgattacagttttaaatccgcctcacaatttgttgagtgggatcaggtcactgcttacctgaacggggttctagtgtggggaaaggaacctggt

SEQ ID NO: 9 - DNA, 12 bp, Artificial Sequence
  HDEL
catgacgagctt

SEQ ID NO: 10 - DNA, 2153 bp, Artificial Sequence
  FULL EXPRESSION CASSETTE (FULL SEQUENCE): BIP_M_GCCAHa3 _CBM3_HDEL
tctagaattattacatcaaaacaaaaaatggctcgctcgtttggagctaacagtaccgttgtgttggcgatcatcttcttcggtgagtgattttccgatcttcttctccgatttagatctcctctacattgttgcttaatctcagaaccttttttcgttgttcctggatctgaatgtgtttgtttgcaatttcacgatcttaaaaggttagatctcgattggtattgacgattggaatctttacgatttcaggatgtttatttgcgttgtcctctgcaatagaagaggctacgaagttaaggatcccgatggcaaacatcactgtggattacttatataacaaggaaactaaattatttacagcaaagctaaatgttaatgagaatgtggaatgtggaaacaatacttgcacaaacaatgaggtgcataaccttacagaatgtaaaaatgcgtctgtttccatatctcataattcatgtactgctcctgatggtggaggaggttctggtggtggatcaactagtcatattaatttgaaagtgaagggacaggacggaaacgaggttttcttccgtatcaaaagatcaacacaactcaagaaactcatgaatgcttactgcgatagacaaagcgtggacatgacagctatagctttcctatttgatgggagaaggttgagagcggaacagactccggatgagcttgaaatggaagatggagatgagattgacgcaatgttacatcagactggtgccggcggtcccgggggtatgaacttcttcgctaccgcctccgtctttctactcttcttgtccgtcgccctccccgtgcgggcgaacgaggaaatcgaggtcgacaccgccggctgccccgtcaagagcgcccaaggagacttcagttatgacatgactcttccaaacaaccccacccgctggggcgacatcaaggaggacttcgccacatgcaaggaaggagaaaagcaatcgcccatcaacttccccgccaacgttcaatacgccccgaaatcggccggacccaagtctcaaatgtcgctcgcaaacatgacctttggcgcctcctcctacaactgggccatgtcctgcagcgacgaatccggatcgtgtggaaagacctccttcgctggaaagacctatgaacttatcaatgttcacttccactccccgagtgagcacaagttgttcggcaaagaatatccgcttgaatgtcacatggtgcatgctgccgaggatggatcgcttgctgtggtcggaatgatgtttgagtacgccgaacaaacctcctatcccgccagaatttaccagaacgtcgttgaggaatatggcgacaacgtcgtcttttccactattttgggaggcgtcaagagcgatcgtggagaatgggctgtgccggtgggtcaactggtcaaccataacaagggatattgctcctactccgggtcgctcaccacaccgccttgcactgaaagtgtcacctggttcatgtctatgaacatctggaccgtgtctgaacgacaggtgcatgactacgtccgaacggttggcaccagcattgagggaaatcatcgaccggttcaaccactcaacgaacgtccggtcacttgctacgtgtcctaaggaggaggttcaggtggtaccgtatcaggtaaccttaaggtggagttttacaactcgaacccttctgatacaactaactcaataaacccacagttcaaagttacaaacacaggcagctctgcgatcgatttgtctaaattaaccctcagatactattatacggttgatggacagaaggaccagactttctggtgtgatcatgcagctatcattggttctaacggtagctacaacggaattacatcaaacgtgaagggcactttcgttaagatgtcctctagcactaacaacgcagacacatatttggagatcagttttacggggggaacccttgaaccaggtgctcacgtccagattcaaggaagattcgctaaaaacgactggtcgaactatacccaaagtaatgattacagttttaaatccgcctcacaatttgttgagtgggatcaggtcactgcttacctgaacggggttctagtgtggggaaaggaacctggtcatgacgagctttaactcgag

SEQ ID NO: 11 - protein, 254 aa, Artificial Sequence
  AMINO ACID SEQUENCE OF SAZCA
MKKFILSILSLSIVSIAGEHAILQKNAEVHHWSYEGENGPENWAKLNPEYFWCNLKNQSPVDISDNYKVHAKLEKLHINYNKAVNPEIVNNGHTIQVNVLEDFKLNIKGKEYHLKQFHFHAPSEHTVNGKYYPLEMHLVHKDKDGNIAVIGVFFKEGKANPELDKVFKNALKEEGSKVFDGSININALLPPVKNYYTYSGSLTTPPCTEGVLWIVLKQPITASKQQIELFKSIMKHNNNRPTQPINSRYILESN

SEQ ID NO: 12 - DNA, 761 bp, Artificial Sequence
  BACTERIAL CARBONIC ANHYDRASE (SAZCA) FROM SULFURIHYDROGENIBIUM AZORENSE
atgaaaaaattcatactgagcatactcagtctatccatcgtctcaatagcgggagagcatgccattctgcaaaaaaatgcagaggtacatcactggtcatatgaaggtgaaaacggtccagagaattgggcaaaattgaacccggaatatttttggtgcaacctgaagaatcagtctcccgtggatatatctgacaattataaggtgcacgcaaagctggaaaaattgcatatcaactacaataaagcagtcaatcctgagatagtgaataatgggcacacaattcaggtgaatgtccttgaggactttaagctaaatataaaaggaaaagagtatcatctcaaacagttccatttccatgcaccgagtgaacacaccgtcaacggaaaatactatcccttggagatgcacctggtacataaagataaagacggtaacatcgctgtcatcggggttttttttaaggaaggtaaggcgaacccagaactcgataaagtcttcaaaaacgccctgaaggaagagggctctaaggtcttcgacggaagtataaacatcaacgctttacttccgcccgtgaagaactactatacgtacagcggctcactgacaactccgccgtgcactgaaggagttttatggattgtactgaagcagccgattaccgcttccaagcagcaaatagaactctttaagtcaataatgaagcataataacaatcgacccacgcaacctatcaatagccgatacatcttggaatctaa

SEQ ID NO: 13 - DNA, 1805 bp, Artificial Sequence
  FULL EXPRESSION CASSETTE (FULL SEQUENCE): BIP_M_SAZCA_CBM3_HDEL
tctagaattattacatcaaaacaaaaaatggctcgctcgtttggagctaacagtaccgttgtgttggcgatcatcttcttcggtgagtgattttccgatcttcttctccgatttagatctcctctacattgttgcttaatctcagaaccttttttcgttgttcctggatctgaatgtgtttgtttgcaatttcacgatcttaaaaggttagatctcgattggtattgacgattggaatctttacgatttcaggatgtttatttgcgttgtcctctgcaatagaagaggctacgaagttaaggatcccgatggcaaacatcactgtggattacttatataacaaggaaactaaattatttacagcaaagctaaatgttaatgagaatgtggaatgtggaaacaatacttgcacaaacaatgaggtgcataaccttacagaatgtaaaaatgcgtctgtttccatatctcataattcatgtactgctcctgatggtggaggaggttctggtggtggatcaactagtatgaaaaaattcatactgagcatactcagtctatccatcgtctcaatagcgggagagcatgccattctgcaaaaaaatgcagaggtacatcactggtcatatgaaggtgaaaacggtccagagaattgggcaaaattgaacccggaatatttttggtgcaacctgaagaatcagtctcccgtggatatatctgacaattataaggtgcacgcaaagctggaaaaattgcatatcaactacaataaagcagtcaatcctgagatagtgaataatgggcacacaattcaggtgaatgtccttgaggactttaagctaaatataaaaggaaaagagtatcatctcaaacagttccatttccatgcaccgagtgaacacaccgtcaacggaaaatactatcccttggagatgcacctggtacataaagataaagacggtaacatcgctgtcatcggggttttttttaaggaaggtaaggcgaacccagaactcgataaagtcttcaaaaacgccctgaaggaagagggctctaaggtcttcgacggaagtataaacatcaacgctttacttccgcccgtgaagaactactatacgtacagcggctcactgacaactccgccgtgcactgaaggagttttatggattgtactgaagcagccgattaccgcttccaagcagcaaatagaactctttaagtcaataatgaagcataataacaatcgacccacgcaacctatcaatagccgatacatcttggaatctaatggaggaggttcaggtggtaccgtatcaggtaaccttaaggtggagttttacaactcgaacccttctgatacaactaactcaataaacccacagttcaaagttacaaacacaggcagctctgcgatcgatttgtctaaattaaccctcagatactattatacggttgatggacagaaggaccagactttctggtgtgatcatgcagctatcattggttctaacggtagctacaacggaattacatcaaacgtgaagggcactttcgttaagatgtcctctagcactaacaacgcagacacatatttggagatcagttttacggggggaacccttgaaccaggtgctcacgtccagattcaaggaagattcgctaaaaacgactggtcgaactatacccaaagtaatgattacagttttaaatccgcctcacaatttgttgagtgggatcaggtcactgcttacctgaacggggttctagtgtggggaaaggaacctggtcatgacgagctttaactcgag